European Patent Specification EP 3 730 515 B1, published July 26, 2023. Title: A fully-human T-cell receptor specific for the 369-377 epitope derived from the Her2/Neu (ERBB2) receptor protein. Applicant: The Trustees of the University of Pennsylvania. Application not yet assigned. The sequence listing filed with the application follows.

SEQUENCE LISTING (9 sequences)

SEQ ID NO: 1 - DNA, 810 bp, Homo sapiens
atggcctctgcacccatctcgatgcttgcgatgctcttcacattgagtgggctgagagctcagtcagtggctcagccggaagatcaggtcaacgttgctgaagggaatcctctgactgtgaaatgcacctattcagtctctggaaacccttatcttttttggtatgttcaataccccaaccgaggcctccagttccttctgaaatacatcacaggggataacctggttaaaggcagctatggctttgaagctgaatttaacaagagccaaacctccttccacctgaagaaaccatctgcccttgtgagcgactccgctttgtacttctgtgctgtggaagatgccagactcatgtttggagatggaactcagctggtggtgaagcccaatatccagaaccctgaccctgccgtgtaccagctgagagactctaaatccagtgacaagtctgtctgcctattcaccgattttgattctcaaacaaatgtgtcacaaagtaaggattctgatgtgtatatcacagacaaaactgtgctagacatgaggtctatggacttcaagagcaacagtgctgtggcctggagcaacaaatctgactttgcatgtgcaaacgccttcaacaacagcattattccagaagacaccttcttccccagcccagaaagttcctgtgatgtcaagctggtcgagaaaagctttgaaacagatacgaacctaaactttcaaaacctgtcagtgattgggttccgaatcctcctcctgaaagtggccgggtttaatctgctcatgacgctgcggctgtggtccagc

SEQ ID NO: 2 - protein, 270 aa, Homo sapiens
MASAPISMLAMLFTLSGLRAQSVAQPEDQVNVAEGNPLTVKCTYSVSGNPYLFWYVQYPNRGLQFLLKYITGDNLVKGSYGFEAEFNKSQTSFHLKKPSALVSDSALYFCAVEDARLMFGDGTQLVVKPNIQNPDPAVYQLRDSKSSDKSVCLFTDFDSQTNVSQSKDSDVYITDKTVLDMRSMDFKSNSAVAWSNKSDFACANAFNNSIIPEDTFFPSPESSCDVKLVEKSFETDTNLNFQNLSVIGFRILLLKVAGFNLLMTLRLWSS

SEQ ID NO: 3 - DNA, 936 bp, Homo sapiens
atgggcttcaggctcctctgctgtggtgccttctgcctcctccaagcaggtcccttggacacagctgtttcccagactccaaaatacctggtcacacagatgggaaacgacaagtccattaaatgtgaacaaaatctgggccatgatactatgtattggtataaacaggactctaagaaatttctgaagataatgtttagctacaataataaggagctcattataaatgaaacagttccaaatcgcttctcacctaaatctccagacaaagctcacttaaatcttcacatcaattccctggagcttggtgactctgctgtgtatttctgtgccagcagccaactagcggactacaatgagcagttcttcgggccagggacacggctcaccgtgctagaggacctgaaaaacgtgttcccacccgaggtcgctgtgtttgagccatcagaagcagagatctcccacacccaaaaggccacactggtgtgcctggccacaggcttctaccccgaccacgtggagctgagctggtgggtgaatgggaaggaggtgcacagtggggtcagcacagacccgcagcccctcaaggagcagcccgccctcaatgactccagatactgcctgagcagccgcctgagggtctcggccaccttctggcagaacccccgcaaccacttccgctgtcaagtccagttctacgggctctcggagaatgacgagtggacccaggatagggccaaacctgtcacccagatcgtcagcgccgaggcctggggtagagcagactgtggcttcacctccgagtcttaccagcaaggggtcctgtctgccaccatcctctatgagatcttgctagggaaggccaccttgtatgccgtgctggtcagtgccctcgtgctgatggctatggtcaagagaaaggattccagaggctag

SEQ ID NO: 4 - protein, 311 aa, Homo sapiens
MGFRLLCCGAFCLLQAGPLDTAVSQTPKYLVTQMGNDKSIKCEQNLGHDTMYWYKQDSKKFLKIMFSYNNKELIINETVPNRFSPKSPDKAHLNLHINSLELGDSAVYFCASSQLADYNEQFFGPGTRLTVLEDLKNVFPPEVAVFEPSEAEISHTQKATLVCLATGFYPDHVELSWWVNGKEVHSGVSTDPQPLKEQPALNDSRYCLSSRLRVSATFWQNPRNHFRCQVQFYGLSENDEWTQDRAKPVTQIVSAEAWGRADCGFTSESYQQGVLSATILYEILLGKATLYAVLVSALVLMAMVKRKDSRG

SEQ ID NO: 5 - DNA, 1827 bp, Homo sapiens
atggcctctgcacccatctcgatgcttgcgatgctcttcacattgagtgggctgagagctcagtcagtggctcagccggaagatcaggtcaacgttgctgaagggaatcctctgactgtgaaatgcacctattcagtctctggaaacccttatcttttttggtatgttcaataccccaaccgaggcctccagttccttctgaaatacatcacaggggataacctggttaaaggcagctatggctttgaagctgaatttaacaagagccaaacctccttccacctgaagaaaccatctgcccttgtgagcgactccgctttgtacttctgtgctgtggaagatgccagactcatgtttggagatggaactcagctggtggtgaagcccaatatccagaaccctgaccctgccgtgtaccagctgagagactctaaatccagtgacaagtctgtctgcctattcaccgattttgattctcaaacaaatgtgtcacaaagtaaggattctgatgtgtatatcacagacaaaactgtgctagacatgaggtctatggacttcaagagcaacagtgctgtggcctggagcaacaaatctgactttgcatgtgcaaacgccttcaacaacagcattattccagaagacaccttcttccccagcccagaaagttcctgtgatgtcaagctggtcgagaaaagctttgaaacagatacgaacctaaactttcaaaacctgtcagtgattgggttccgaatcctcctcctgaaagtggccgggtttaatctgctcatgacgctgcggctgtggtccagccgggccaagcggtccggatccggagccaccaacttcagcctgctgaagcaggccggcgacgtggaggagaaccccggccccatgggcttcaggctcctctgctgtggtgccttctgcctcctccaagcaggtcccttggacacagctgtttcccagactccaaaatacctggtcacacagatgggaaacgacaagtccattaaatgtgaacaaaatctgggccatgatactatgtattggtataaacaggactctaagaaatttctgaagataatgtttagctacaataataaggagctcattataaatgaaacagttccaaatcgcttctcacctaaatctccagacaaagctcacttaaatcttcacatcaattccctggagcttggtgactctgctgtgtatttctgtgccagcagccaactagcggactacaatgagcagttcttcgggccagggacacggctcaccgtgctagaggacctgaaaaacgtgttcccacccgaggtcgctgtgtttgagccatcagaagcagagatctcccacacccaaaaggccacactggtgtgcctggccacaggcttctaccccgaccacgtggagctgagctggtgggtgaatgggaaggaggtgcacagtggggtcagcacagacccgcagcccctcaaggagcagcccgccctcaatgactccagatactgcctgagcagccgcctgagggtctcggccaccttctggcagaacccccgcaaccacttccgctgtcaagtccagttctacgggctctcggagaatgacgagtggacccaggatagggccaaacctgtcacccagatcgtcagcgccgaggcctggggtagagcagactgtggcttcacctccgagtcttaccagcaaggggtcctgtctgccaccatcctctatgagatcttgctagggaaggccaccttgtatgccgtgctggtcagtgccctcgtgctgatggctatggtcaagagaaaggattccagaggctag

SEQ ID NO: 6 - protein, 272 aa, Homo sapiens
MASAPISMLAMLFTLSGLRAQSVAQPEDQVNVAEGNPLTVKCTYSVSGNPYLFWYVQYPNRGLQFLLKYITGDNLVKGSYGFEAEFNKSQTSFHLKKPSALVSDSALYFCAVEDARLMFGDGTQLVVKPNIQNPDPAVYQLRDSKSSDKSVCLFTDFDSQTNVSQSKDSDVYITDKTVLDMRSMDFKSNSAVAWSNKSDFACANAFNNSIIPEDTFFPSPESSCDVKLVEKSFETDTNLNFQNLSVIGFRILLLKVAGFNLLMTLRLWSSRA

SEQ ID NO: 7 - protein, 312 aa, Homo sapiens
PMGFRLLCCGAFCLLQAGPLDTAVSQTPKYLVTQMGNDKSIKCEQNLGHDTMYWYKQDSKKFLKIMFSYNNKELIINETVPNRFSPKSPDKAHLNLHINSLELGDSAVYFCASSQLADYNEQFFGPGTRLTVLEDLKNVFPPEVAVFEPSEAEISHTQKATLVCLATGFYPDHVELSWWVNGKEVHSGVSTDPQPLKEQPALNDSRYCLSSRLRVSATFWQNPRNHFRCQVQFYGLSENDEWTQDRAKPVTQIVSAEAWGRADCGFTSESYQQGVLSATILYEILLGKATLYAVLVSALVLMAMVKRKDSRG

SEQ ID NO: 8 - protein, 1255 aa, Homo sapiens [sequence omitted]

SEQ ID NO: 9 - protein, 9 aa, Homo sapiens
KIFGSLAFL